European Patent Application EP 4 647 497 A1, published November 12, 2025. Title: Manganese influx protein activity-modulated recombinant microorganism and method for producing O-phosphoserine, cysteine and its derivatives using the same. Applicant: CJ CheilJedang Corporation. The sequence listing filed with the application follows.

SEQUENCE LISTING (59 sequences)

SEQ ID NO: 1 - protein, 412 aa, Escherichia sp.
MTNYRVESSSGRAARKMRLALMGPAFIAAIGYIDPGNFATNIQAGASFGYQLLWVVVWANLMAMLIQILSAKLGIATGKNLAEQIRDHYPRPVVWFYWVQAEIIAMATDLAEFIGAAIGFKLILGVSLLQGAVLTGIATFLILMLQRRGQKPLEKVIGGLLLFVAAAYIVELIFSQPNLAQLGKGMVIPSLPTSEAVFLAAGVLGATIMPHVIYLHSSLTQHLHGGSRQQRYSATKWDVAIAMTIAGFVNLAMMATAAAAFHFSGHTGVADLDEAYLTLQPLLSHAAATVFGLSLVAAGLSSTVVGTLAGQVVMQGFIRFHIPLWVRRTVTMLPSFIVILMGLDPTRILVMSQVLLSFGIALALVPLLIFTSDSKLMGDLVNSKRVKQTGWVIVVLVVALNIWLLVGTALGL

SEQ ID NO: 2 - DNA, 1239 bp, Escherichia coli
  source 1..1239: mol_type = genomic DNA
atgacgaactatcgcgttgagagtagcagcggacgggcggcgcgcaagatgaggctcgcattaatgggacctgcgttcattgcggcgattggttatatcgatcccggtaactttgcgaccaatattcaggcgggtgctagcttcggctatcagctactgtgggttgtcgtttgggccaacctgatggcgatgctgattcagatcctctctgccaaactagggattgccaccggtaaaaatctggcggagcagattcgcgatcactatccgcgtcccgtagtgtggttctattgggttcaggcagaaattattgcgatggcaaccgacctggcggaatttattggtgcggcgatcggttttaaactcattcttggtgtttcgttgttgcagggcgcggtgctgacggggatcgcgactttcctgattttaatgctgcaacgtcgcgggcaaaaaccgctggagaaagtgattggcgggttactgttgtttgttgccgcggcttacattgtcgagttgattttctcccagcctaacctggcgcagctgggtaaaggaatggtgatcccgagtttacctacttcggaagcggtcttcctggcagcaggcgtgttaggggcgacgattatgccgcatgtgatttatttgcactcctcgctcactcagcatttacatggcggttcgcgtcaacaacgttattccgccaccaaatgggatgtggctatcgccatgactattgccggttttgtcaatctggcgatgatggctacagctgcggcggcgttccacttttccggtcatactggtgttgccgatcttgatgaggcttatctgacgctgcaaccgctgttaagccacgctgcggcaacggtctttggattaagcctggttgctgcggggctgtcttcaacggtggtggggacactggcggggcaggtggtgatgcagggcttcattcgctttcatatcccgctgtgggtgcgtcgtacagtcaccatgttgccgtcatttattgtcattctgatgggattagatccgacacggattctggttatgagtcaggtactgttaagttttggtatcgctctggcgctggttccactgctgattttcaccagtgacagcaagttgatgggcgatctggtgaacagcaaacgcgtaaaacagacaggctgggtgattgtggtgctggtcgtggcgctgaatatctggttgttggtggggacggcgctgggattgtag

SEQ ID NO: 3 - DNA, 15655 bp, unidentified
  source 1..15655: mol_type = genomic DNA
tcgacggacgatagataattcctgagacaatagtgtaaaaaacgagccgctgggggtgttttaaaccccagcggcttttttttagtaaaaatccttcatcgcatagtgcagaacgtacaaaactgttcatttttcaaccaccagagattcacgtcccgaacgcacaaataatcgcctgaaaaaaatcacctgctacaatgatgttaaaaaatacgtaaatttgttgctgcgtttttgttatggaatgacaaaagcgtgtcacagatcaagaaaatactctcttttggggggaggaatcgacacaaattcctgtcaaaatagacccgtattttttccattgcttcacaacggacacgattcaacaacatctaattatcctggagtcgtcaaggatctggggtgaaagggcattaaatgctaatggtgttgatattatgtaaactaatgtgaagaaacttttgttaaagttgacaaaaggttatagaaaggagtaaaaaaccacatcaattagctgtataaaagaatttctacagtgattgtaaggttttttttattcctccccatgaatcgatgtggcgtccatctgccgtgaagagcagtgaatctggcgctacttttgatgagtaagcaatgagtatgtcaacatccactgaagtcatcgctcatcactgggcattcgctatctttcttatcgttgccattggcctgtgttgcctgatgctggtaggcggttggtttttaggcggtcgcgcacgcgcgaggtcgaaaaacgtgccgtttgaatccggtatcgactcggtcggctccgcccgcttacgcctgtccgccaagttttatctggtggccatgttcttcgttatcttcgacgttgaagcgctgtatctgttcgcatggtcaacctctatccgcgaaagcggctgggtaggctttgtggaagctgcaatttttatttttgtgttactggcaggtctggtttatctggtgcgtattggcgcgctggactggacgcccgcgcgttcacgccgcgagcgtatgaacccggaaacgaacagtatcgctaatcgtcaacgctaaccgcgaggcattaagatggattatacgctcacccgcatagatcccaacggtgagaacgaccgttaccccctgcaaaagcaggagatcgtaaccgaccctctggagcaagaagttaacaaaaacgtgtttatgggcaagctcaatgacatggttaactggggtcgtaaaaactcaatttggccgtataacttcggtctttcctgctgttacgttgagatggtgacttcgtttaccgcggtgcatgacgtggcgcgttttggcgcagaagtattgcgtgcttcgccgcgtcaggctgacctgatggtggttgcaggaacctgctttaccaaaatggcaccggttattcagcgtctgtatgaccagatgctggaaccaaaatgggttatctcaatgggtgcctgtgccaactctggtggtatgtacgatatttattccgttgtgcagggcgtcgataaattcatcccggttgatgtgtatatcccgggctgcccgccgcgtcctgaagcgtacatgcaggcactgatgctgttgcaggaatctatcggcaaagaacgtcgtccgctctcctgggtggttggcgatcagggcgtttatcgcgccaatatgcaatcagagcgcgaacgcaagcgcggtgaacgcattgccgtaactaacctgcgtacacctgacgagatttaatttgcgcctgtcggcaaagggatttttcttcgcttattcctaaatctatttcgcgaagcttactgcgccgacagtcaccacggaccatttgcaatggtgaacaatatgaccgacttaaccgcgcaagaacccgcctggcagacccgcgatcatcttgatgatccggtgattggcgaactgcgcaaccgttttgggccggatgcctttactgttcaggcgactcgcaccggggttcccgttgtgtggatcaagcgtgaacaattactggaagttggcgatttcttaaagaaactgccgaaaccttacgtcatgctgtttgacttacacggcatggacgaacgtctgcgcacacaccgcgaagggttacctgccgcggatttttccgttttctaccatctgatttctatcgatcgtaaccgcgacatcatgctgaaggtggcgctggcagaaaacgacctgcacgtaccgaccttcaccaaactgttcccgaacgctaactggtatgagcgtgaaacctgggatctgtttggcattactttcgacggtcacccgaacctgcgacgcatcatgatgccgcaaacctggaaaggtcacccgctgcgtaaagattatccggcgcgcgctaccgaattctcgccgtttgagctgaccaaagccaaacaggatctggagatggaagccctgaccttcaaaccggaagagtgggggatgaagcgcggcaccgaaaacgaggacttcatgttcctcaacctcggtccgaaccacccgtcggcgcacggggctttccgtatcgttttgcaactcgatggcgaagagattgtcgactgcgtaccagacatcggttaccaccaccgtggtgcggagaaaatgggcgaacgccagtcctggcacagctacattccgtatactgaccgtatcgaatacctcggcggctgcgttaacgaaatgccttacgtgctggcggtagagaaactggccgggatcaccgtgccggatcgcgttaacgtcattcgcgttatgctctccgaactgttccgcatcaacagtcacctgctgtatatctcgacctttattcaggacgtcggcgcaatgacgccagtgttcttcgcctttaccgatcgtcagaaaatttacgatctggtggaagcaatcactggtttccgtatgcacccggcgtggttccgtattggcggcgtagcgcacgacctgccgcgcggctgggatcgcctgctgcgtgagttcctcgactggatgccgaaacgtctggcgtcttacgagaaagcggcgctgcaaaacaccattctgaaaggtcgttcccagggcgttgccgcctatggcgcgaaagaggcgctggagtggggcaccactggcgcgggcctgcgtgctaccgggatcgacttcgacgtgcgtaaggcgcgtccttattctggctatgaaaacttcgactttgaaatcccggtgggtggtggcgtttctgactgctacacccgcgtaatgcttaaagtggaagagctgcgccagagtctgcgcattcttgagcagtgcctcaacaacatgccggaaggcccgttcaaagcggatcacccgctgaccacgccgccgccgaaagagcgcacgctgcaacatatcgaaaccctgatcacccacttcctgcaagtgtcgtggggtccggtgatgcctgccaatgaatctttccagatgattgaggcgaccaaagggatcaacagttactacctgaccagcgacggcagcaccatgagttaccgcacccgtgttcgtaccccgagctttgcgcatttgcagcaaattccggcggcgatccgcggcagcctggtgtctgacctgattgtttatctgggcagtatcgattttgttatgtcagatgtggaccgctaattatgcacgagaatcaacaaccacaaaccgaggcttttgagctgagtgcggcagagcgtgaagcgatcgagcacgagatgcaccactacgaagacccgcgtgcggcgtccattgaagcgctgaaaatcgttcagaagcagcgtggctgggtgccggatggtgcgatccacgcgatcgccgatgtgctgggtattccggcaagcgacgtcgaaggtgtggcaacgttctacagtcagatcttccgccagccggttggtcgccatgtgatccgttattgtgacagcgtggtctgtcatatcaacggttatcagggtattcaggcggcgctcgagaaaaagctgaacatcaaaccagggcaaacgacatttgatggccgctttacgctgctgccaacttgctgcctggggaactgtgataaagggccaaacatgatgatcgatgaggacactcacgcgcatctgaccccggaagcgatccctgaactgctggagcggtataaatgaaaaacattatccgtactcccgaaacgcatccgctgacctggcgtctgcgcgatgacaaacagccagtgtggctggacgaataccgcagcaaaaacggttacgaaggcgcgcgtaaggcgctgaccgggctgtctccggacgaaatcgttaatcaggtaaaagacgctggtctgaaagggcgcggcggcgcgggcttctcgactggcctgaaatggagcctgatgccgaaagacgaatccatgaacatccgttacctgctgtgtaatgccgatgaaatggagccgggcacctataaagaccgcctgttgatggagcaactgccgcacctgctggtggaaggtatgctcatctccgcgtttgcgctgaaagcttaccgtggctacatcttcctgcgtggcgaatatatcgaagcggcagttaatctgcgccgtgccattgccgaagccaccgaagcgggtctgcttggcaaaaacattatgggaacaggtttcgatttcgaactgttcgtccataccggggcagggcgctacatctgcggggaagaaacagcgttaatcaactccctggaaggacgtcgtgctaacccacgctcgaagccacccttcccggcaacctccggcgcatggggtaaaccgacctgtgtcaacaacgtcgaaaccctgtgtaacgttccggcgatcctcgctaacggcgtggagtggtatcagaacatctcgaaaagtaaagatgctggcaccaagctgatgggcttctccggtcgggtgaaaaatccgggactgtgggaactgccgttcggcaccaccgcacgcgagatcctcgaagattacgccggtggtatgcgtgatggtctgaaatttaaagcctggcagccaggcggcgcggggactgacttcctgaccgaagcgcaccttgatctgccgatggaattcgaaagtatcggtaaagcgggcagccgtctgggtacggcgctggcgatggcggttgaccatgagatcaacatggtgtcgctggtgcgtaacctggaagagtttttcgcccgtgagtcctgcggctggtgtacgccgtgccgcgacggtctgccgtggagcgtgaaaattctgcgtgcgctggagcgtggtgaaggtcagccgggcgatatcgaaacacttgagcaactgtgtcgattcttaggcccgggtaaaactttctgtgcccacgcacctggtgcagtggagccgttacagagcgccatcaaatatttccgcgaagaatttgaggcgggaatcaaacagccgttcagcaatacccatttgattaatgggattcagccgaacctgctgaaagagcgctggtaaccgaatttcgattaacgctcagtctctgactgagaaaactggaagcatgctaatggctacaattcatgtagacggcaaagaatacgaggtcaacggagcggacaacctgctggaagcttgtctgtctctgggccttgatattccttacttttgctggcatccggcgctgggaagtgtcggtgcttgccgccagtgtgcggtgaagcaataccaaaacgcggaagacacgcgtggtcgcctggtgatgtcctgtatgacaccggcttccgatggcacctttatttccattgacgacgaagaagcgaaacagttccgtgaaagcgtggtcgagtggttgatgaccaaccacccgcacgactgtccggtatgtgaagagggcggtaactgccatcttcaggatatgactgtgatgaccggacacagcttccgtcgctaccgtttcaccaaacgtacccaccgtaatcaggatttggggccattcatctctcacgaaatgaaccgctgcatcgcctgctaccgctgtgtgcgttactacaaagattacgctgacggtacagatctgggcgtttacggtgcgcacgacaacgtctacttcggtcgcccggaagacggcacgctggaaagcgaattttccggtaacctggtcgaaatttgcccgaccggcgtatttaccgacaaaacgcactccgagcgttacaaccgtaaatgggatatgcagtttgcgccgagcatctgccagcaatgttccatcggctgtaacatcagccccggtgaacgttacggcgaactgcgtcgtatcgaaaaccgttacaacggtacggtaaaccactacttcctctgcgaccgtggtcgtttcggttacggttacgtcaacctgaaggatcgtccgcgtcagccagtacagcgtcgtggcgatgatttcattaccctcaacgccgaacaggcaatgcagggcgcggcagatattctgcgtcagtcgaagaaagtgatcggtattggttctccgcgtgccagcgtggaaagcaactttgcgctgcgtgaactggtgggcgaagaaaacttctacaccggtatcgctcacggtgagcaggaacgtctgcaactggcgctgaaagtgctgcgtgaaggcggcatttatactccggctctgcgcgaaatcgaatcttacgatgcggtactggtgctgggcgaagacgttacccagaccggcgcgcgcgtcgcgctggcagtgcgtcaggctgtgaaaggtaaagcgcgcgaaatggcggcagcacagaaagtggctgactggcagattgcggcaatcctcaacatcggtcaacgtgcgaagcatccgctgtttgttaccaacgttgatgacacccgtctggatgatatcgcggcgtggacttaccgcgcaccggttgaagatcaggcgcgtttaggttttgccatcgcccatgcgctggataactctgcaccagcggttgacggtatcgaacctgagctgcaaagcaaaatcgacgtcatcgtgcaggcactggcaggtgcgaagaaaccgttgattatctccgggacgaacgccggtagcttagaggtgattcaggcggcggctaacgtcgcgaaagccctgaaaggtcgcggcgctgacgtcggtatcaccatgattgcccgttccgtcaacagcatggggctgggcattatgggtggcggttcgcttgaagaagcgttaaccgaactggaaaccggacgcgccgacgcggtggtggtgttggaaaacgatctgcatcgtcacgcttctgctatccgcgtgaatgctgcgctggctaaagcaccgctggtgatggtggttgatcatcaacgcacagcgattatggaaaacgcccatctggtactttctgctgccagctttgctgaaagcgacggtacggtgatcaacaacgaaggccgcgcccaacgtttcttccaggtttacgatcctgcttattacgacagcaaaactgtcatgctggaaagctggcgctggttacactcgctgcacagcaccctgctgagccgtgaagtggactggacgcagctcgaccatgtgattgacgctgttgtggcgaaaatcccggaactggcaggtatcaaagatgctgcgccggatgcgacattccgtattcgtgggcagaaactggcccgtgaaccgcaccgttacagcggtcgtaccgccatgcgcgccaatatcagcgttcatgagccgcgtcagccgcaggatattgacaccatgttcaccttctcgatggaaggtaacaaccagccgactgcgcaccgttcgcaagtgccgtttgcctgggcgccgggctggaactccccgcaggcgtggaacaaattccaggacgaagtgggcggcaaactgcgctttggcgatccgggcgtgcgtctgtttgaaaccagcgaaaatggtctggattacttcaccagcgtaccggcacgcttccagccgcaggacgggaaatggcgtatcgcgccgtattaccacctgtttggcagcgatgaattgtcacagcgtgctccggtcttccagagccgtatgccgcagccgtacatcaaactcaacccagcggatgccgcgaagttgggtgtgaacgcaggtacacgcgtctcctttagttacgatggcaacacggtcacgctgccggttgaaatcgccgaaggactgacggcagggcaggtgggcttgccgatgggtatgtccggcattgctccggtgctggctggcgcgcatcttgaggatctcaaggaggcacaacaatgagttggatatcaccggaactgattgagatcctgctgaccatcctcaaagcggtggtgatcctgctggtggttgtcacctgcggggcattcatgagctttggcgaacgtcgcctgctgggtctgttccagaaccgttacggacctaaccgtgttggctggggcggttcgctccagctggttgcggacatgatcaaaatgttctttaaagaagactggatcccgaaattctcggatcgcgtcatctttaccctggcaccgatgattgcctttacctcgctgctgctggcctttgcgattgtgccagtcagtccgggttgggtggttgccgacctgaacatcgggattttgttcttcctgatgatggcaggtctggcggtttacgcggtgctgtttgcgggctggtcaagtaacaacaaatactcgttgctgggtgcgatgcgtgcttctgcgcagaccctgagctacgaagtgttcctcgggctttccttgatgggcgtggtggcgcaggccggttcattcaacatgaccgacatcgtcaacagccaggcgcatgtgtggaacgttatcccgcaattctttggttttattacctttgccatcgcgggcgtggcggtatgtcaccgtcacccgtttgaccagccggaagccgagcaggaactggcggatggttaccacattgaatattccggtatgaagttcggtctgttcttcgtgggtgagtacatcgggattgtgaccatctctgcattgatggtgacgctgttcttcggtggctggcaaggcccgttgttaccgccattcatctggttcgcgctgaaaaccgcgttctttatgatgatgttcattttgattcgtgcgtcgttaccgcgtccgcgttatgaccaggtaatgtccttcggctggaaaatctgcctgccgctgacgctgatcaacttgctggtaacggcggctgtcattctctggcaggcgcaataaggggcaataagaccatgaccttaaaagaattgttagtaggtttcggcacccaggttcgtagtatctggatgatcggcctgcacgcgttcgccaaacgcgaaacgcgaatgtacccggaagagccggtctatctgccgccccgttatcgtggtcgtatcgttctgacccgcgacccggacggcgaagagcgttgcgtagcctgtaacctctgcgcggtagcctgcccggtcggctgtatctcgctgcaaaaagcagaaaccaaagacggtcgctggtacccggaatttttccgcatcaacttctcacgctgcattttctgtggtctgtgcgaagaagcctgtccgaccacggcgattcagttaaccccggatttcgaaatgggggaatacaagcgccaggatctggtttacgagaaagaggatctgctgatctccggtccgggcaaatacccggaatataacttctaccggatggcaggtatggcaatcgacggcaaagataagggcgaagcagagaacgaagccaagcctatcgacgtcaagagcctgttaccgtaaggagaggggcaatggagttcgctttttatatctgtggcctgatagccatacttgcgaccttgcgagtgatcacccataccaatccggtacacgcactgctgtacctgattatttcgctgctggcgatttccggggtgttcttctcactgggcgcttacttcgccggtgcgctggaaattatcgtctacgcgggtgccattatggtgctgttcgtgttcgtggtgatgatgctcaacctgggcggttcagaaatcgaacaggaacgccagtggctgaaaccgcaggtgtggattggtccggcaattttgtcggccatcatgctggtggtgattgtttacgccatcctcggtgttaacgatcagggtatcgacggtacgccaatcagtgctaaagcagtgggtattacgctgttcgggccttacgtactggcggtggaactggcttctatgctgctgctcgcaggtctggttgtggccttccacgtcggtcgtgaagagcgtgcgggtgaagtgctgagcaatcgtaaagacgacagcgcgaaaagaaaaacggaggagcacgcatgatccccttacaacatggactgatcctcgcggcaatcttattcgttcttggcttaaccggtctggttatccgtcgcaatctgctgtttatgttgattggtctggaaatcatgattaacgcctccgcgctggccttcgtggtcgccggaagctactggggccagaccgacggtcaggtgatgtacattctcgccatcagcctcgcggcggcagaagcgagtatcggccttgcgctgctgctgcaacttcaccgtcgtcgccagaacctgaacatcgattcagtaagtgagatgcgcggatgaacatgcttgccttaaccattattttgccattgattggcttcgtcctgctggcattctcccgtgggcgctggtctgaaaacgtctcggcgatcgtcggcgtaggctctgtgggcctggcggcgctggtaaccgcctttatcggcgttgatttcttcgctaacggcgagcagacatacagccagccgctgtggacgtggatgtcggtaggcgactttaacatcggttttaacctggtgctggacggcctgtcgctgaccatgctctcggtggtcactggtgtgggtttccttattcacatgtacgcctcctggtatatgcgcggtgaagagggctactctcgcttcttcgcttacaccaacctgttcatcgccagcatggtggttctggtgcttgccgacaacctgctgctgatgtacctcggctgggaaggcgtgggcctgtgctcctatctgctgatcgggttctattacaccgatccgaagaatggcgcagcggcaatgaaagcgttcgtcgtgacccgtgtgggtgacgtgttcctcgctttcgcactgttcattctttacaacgaactgggcaccctgaacttccgcgaaatggtggaactggcaccagcgcactttgctgacggcaataacatgctgatgtgggcgacgctgatgctgctgggcggtgcggtcggtaaatctgcgcagttgccgttgcagacatggcttgccgacgcgatggcgggcccgacgcctgtctccgcgctgatccacgccgcaaccatggtaaccgcgggtgtctacctgatcgcccgtacccacggcctgttcctgatgacgccggaagttctgcatctggtgggtattgtcggggcggttacgctgctgctggccggttttgccgcgctggtacagaccgacatcaaacgtgttctcgcttactctaccatgagccagattggctacatgttcctcgcgcttggcgtgcaggcatgggatgcggcgattttccacttgatgacccacgcgttctttaaagcgctgctgttcctggcatccggttccgtcattctggcctgccatcacgaacagaacatcttcaagatgggcggtctgcgtaaatctattccgctggtttatctctgcttcctggtgggcggcgcagcactgtcggcactaccgctggtcactgcgggcttcttcagtaaggatgagatcctcgcgggtgcgatggcgaatggtcatatcaatctgatggtggcaggtctggtcggtgcgtttatgacctcgctctacaccttccgtatgattttcatcgtcttccacggaaaagaacaaattcacgctcacgccgtgaaaggggtaactcacagcctgccgctgattgtgctgctgatcctttccaccttcgttggcgcactgattgtaccgccgctgcagggcgtgcttccgcaaacgacggaactggcgcacggcagcatgttgaccctggaaattacctctggcgtggtcgcggtggtcggcattctgctggcagcctggctgtggctgggtaaacgtactctggtgacctccatcgccaacagtgcgccgggccgtctgctgggcacctggtggtacaacgcctggggatttgactggctgtatgacaaagtgttcgtcaagccgttcctgggtattgcctggttgctgaaacgcgatccgctgaactcaatgatgaacatcccggctgtcctttcccgctttgcaggtaaaggtctgctgttaagtgagaacggctatctgcgctggtatgtggcatccatgagcatcggtgcggtcgtggtgctggcactgttgatggtactgcgttgagttaaggattgtgggattgcccctgggcatataagaacgtaggtcggataagccgccttcgcggtgcatccgacactacccccagtccgaagagaattttctgtcgtgagaattcgttgaaaatccggtcctgacgggacttttacaaggaataaagatcgccatgttactaccctggctaatattaattccctttattggcggcttcctgtgctggcagaccgaacgctttggcgtcaaggtgccacgctggatcgcgctgatcaccatgggattgacgctggcgctgtcgctgcaactgtggttgcagggcggttattcactgacgcaatccgccggaattccgcagtggcagtctgaattcgacatgccgtggatcccgcgttttggtatctctattcatctcgccattgacgggctgtcgctgctgatggtcgtgctgaccggtctgctcggtgtgctggcggtactatgttcgtggaaagagatcgaaaaatatcagggcttcttccacctcaacctgatgtggatcctgggcggcgttatcggcgtgttccttgccatcgacatgttcctgttcttcttcttctgggaaatgatgctggtgccgatgtacttcctgatcgcactgtgggggcataaagcctctgacggtaaaacgcgtatcacggcggcaaccaagttcttcatttacacccaggcgagtggcctggtgatgttgattgccatcctggcgctggtttttgttcactacaatgcgaccggcgtctggaccttcaactatgaagagctgctgaatacgccaatgtccagtggtgtggaatacctgttaatgctgggcttcttcatcgccttcgcagtcaaaatgccggtggttccgctgcatggctggctgccggatgcgcactcccaggctccgaccgccggttccgttgacctcgcggggatcttgctgaaaactgccgcttacggtttgctgcgtttctccctgccgctgttcccgaacgcgtcggcagagttcgcgccaattgctatgtggctgggtgttatcggcatcttctacggtgcgtggatggccttcgcccagaccgatatcaaacgtctgatcgcctacacctcggtttcccacatgggcttcgtgctgattgctatctacaccggcagccagttggcctaccagggcgcggtaatccagatgattgcgcacggtttgtcggcggcgggtctgtttattctttgtggtcagctttatgaacgtatccatacccgcgacatgcgcatgatgggcggtctgtggagcaagatgaaatggctgccagcactgtcgctgttctttgcggtggcaacgcttgggatgcctggcaccggtaacttcgtcggcgaatttatgattctgttcggcagcttccaggttgtaccggtgattaccgttatctctacctttgggctggtctttgcatctgtttattcgctggcgatgttacatcgcgcttacttcggtaaagcgaaaagccagattgccagccaggaactgccagggatgtcgctgcgtgagctgtttatgatcctgttgctggtggtgctgctggtactgctgggcttctatccgcagccgattctggatacctcgcactccgcgattggcaatatccagcagtggtttgttaattccgttactactacaaggccgtaaatcgccatgacaataactccacaaaacctgatcgcactgctaccgttgctgatcgtcggcttgacggtggtggttgtgatgctctccattgcgtggcgacgcaatcatttcctcaacgctacgctctcggttattgggcttaacgcggcgctggtttcgctctggtttgttggccaggcgggcgctatggacgttacgccgctgatgcgcgttgatggtttcgccatgctttacaccgggctggtattgttggcgagcctcgccacctgtactttcgcctacccgtggcttgaaggctataacgacaacaaggatgagttctacctgttggtgttaattgccgcgctgggcgggatcctgctggcgaatgccaaccatctggcgtctctgttcctcggtatcgaactgatctctttgccgctgtttggcctggtcggttacgctttccgccagaaacgttcactggaagccagtatcaaatacaccatcctttctgccgcagcgtcttctttcctgctgtttggtatggcgctggtgtatgcgcagtctggcgacctgtcgtttgtcgcgttgggtaaaaaccttggcgacggtatgctcaacgagccgctgttgctggcaggtttcggcctgatgattgttggcctcggcttcaaactctctctggtgccgttccacctgtggacgccagacgtataccagggcgcgcctgcgccggtttccactttcctggcgacggcgagcaaaatcgctatcttcggtgtggtgatgcgtctgttcctctacgcaccggtgggtgacagcgaagcgattcgcgtggtgctggcgattatcgcctttgcctccatcatcttcggtaacctgatggcgctgagccagaccaatatcaaacgtctgctcggttactcatctatctctcacctcggctatctgctggtagcgctgattgcgctgcaaaccggcgagatgtcgatggaagcggtaggggtttacctggccggttatctgttcagcagcctcggcgcgttcggcgtggtcagcctgatgtccagcccgtatcgtggcccggatgctgattccctgttctcttaccgcggtctgttctggcatcgtccgatcctcgcggcagtgatgacggtgatgatgctgtctctggccggtatcccgatgacgctgggctttatcggtaagttctacgtgctggcggtcggtgtccaggcacacttgtggtggctggtgggtgccgtggttgtcggttcggcaatcggcctctactactacctgcgcgtggcggtgagcctgtatcttcacgccccggaacaaccgggtcgcgatgcaccatcaaactggcagtacagcgcgggcggtatcgttgtgctgatctctgcactgttggtactggtgctgggtgtatggccacaaccgctgattagcattgtgcgtttggcaatgccgctgatgtaa

SEQ ID NO: 4 - protein, 322 aa, unidentified [sequence omitted]

SEQ ID NO: 5 - DNA, 969 bp, unidentified
  source 1..969: mol_type = genomic DNA
atgcctaacattacctggtgcgacctgcctgaagatgtctctttatggccgggtctgcctctttcattaagtggtgatgaagtgatgccactggattaccacgcaggtcgtagcggctggctgctgtatggtcgtgggctggataaacaacgtctgacccaataccagagcaaactgggtgcggcgatggtgattgttgccgcctggtgcgtggaagattatcaggtgattcgtctggcaggttcactcaccgcacgggctacacgcctggcccacgaagcgcagctggatgtcgccccgctggggaaaatcccgcacctgcgcacgccgggtttgctggtgatggatatggactccaccgccatccagattgaatgtattgatgaaattgccaaactggccggaacgggcgagatggtggcggaagtaaccgaacgggcgatgcgcggcgaactcgattttaccgccagcctgcgcagccgtgtggcgacgctgaaaggcgctgacgccaatattctgcaacaggtgcgtgaaaatctgccgctgatgccaggcttaacgcaactggtgctcaagctggaaacgctgggctggaaagtggcgattgcctccggcggctttactttctttgctgaatacctgcgcgacaagctgcgcctgaccgccgtggtagccaatgaactggagatcatggacggtaaatttaccggcaatgtgatcggcgacatcgtagacgcgcagtacaaagcgaaaactctgactcgcctcgcgcaggagtatgaaatcccgctggcgcagaccgtggcgattggcgatggagccaatgacctgccgatgatcaaagcggcagggctggggattgcctaccatgccaagccaaaagtgaatgaaaaggcggaagtcaccatccgtcacgctgacctgatgggggtattctgcatcctctcaggcagcctgaatcagaagtaa

SEQ ID NO: 6 - protein, 405 aa, unidentified
MPEPVAEPALNGLRLNLRIVSIVMFNFASYLTIGLPLAVLPGYVHDVMGFSAFWAGLVISLQYFATLLSRPHAGRYADSLGPKKIVVFGLCGCFLSGLGYLTAGLTASLPVISLLLLCLGRVILGIGQSFAGTGSTLWGVGVVGSLHIGRVISWNGIVTYGAMAMGAPLGVVFYHWGGLQALALIIMGVALVAILLAIPRPTVKASKGKPLPFRAVLGRVWLYGMALALASAGFGVIATFITLFYDAKGWDGAAFALTLFSCAFVGTRLLFPNGINRIGGLNVAMICFSVEIIGLLLVGVATMPWMAKIGVLLAGAGFSLVFPALGVVAVKAVPQQNQGAALATYTVFMDLSLGVTGPLAGLVMSWAGVPVIYLAAAGLVAIALLLTWRLKKRPPEHVPEAASSS

SEQ ID NO: 7 - DNA, 1218 bp, unidentified
  source 1..1218: mol_type = genomic DNA
atgcccgaacccgtagccgaacccgcgctaaacggattgcgcctgaatttgcgcattgtctctatagtcatgtttaacttcgccagctacctcaccatcgggttgccgctcgctgtattaccgggctatgtccatgatgtgatgggctttagcgccttctgggcaggattggttatcagcctgcaatatttcgccaccttgctgagccgccctcatgccggacgttacgccgattcgctgggacccaaaaagattgtcgtcttcggtttatgcggctgctttttgagcggtctggggtatctgacggcaggattaaccgccagtctgcctgtcatcagcctgttattactttgcctggggcgcgtcatccttgggattgggcaaagttttgccggaacgggatcgaccctatggggcgttggcgtggttggctcgctgcatatcgggcgggtgatttcgtggaacggcattgtcacttacggggcgatggcgatgggtgcgccgttaggcgtcgtgttttatcactggggcggcttgcaggcgttagcgttaatcattatgggcgtggcgctggtggccattttgttggcgatcccgcgtccgacggtaaaagccagtaaaggcaaaccgctgccgtttcgcgcggtgcttgggcgcgtctggctgtacggtatggcgctggcactggcttccgccggatttggcgtcatcgccacctttatcacgctgttttatgacgctaaaggttgggacggtgcggctttcgcgctgacgctgtttagctgtgcgtttgtcggtacgcgtttgttattccctaacggcattaaccgtatcggtggcttaaacgtagcgatgatttgctttagcgttgagataatcggcctgctactggttggcgtggcgactatgccgtggatggcgaaaatcggcgtcttactggcgggggccgggttttcgctggtgttcccggcattgggtgtagtggcggtaaaagcggttccgcagcaaaatcagggggcggcgctggcaacttacaccgtatttatggatttatcgcttggcgtgactggaccactggctgggctggtgatgagctgggcgggcgtaccggtgatttatctggcggcggcgggactggtcgcaatcgcgttattactgacgtggcgattaaaaaaacggcctccggaacacgtccctgaggccgcctcatcatcttaa

SEQ ID NO: 8 - DNA, 300 bp, synthetic construct
  source 1..300: mol_type = other DNA
caggaagccgcttctattgcacaagagataaagcgtctaccttaattataaagatttgtaaatataaccgtctccggtatgttgcctgaggcggtttttttgtctctaacgtgcggaaaaatttgttcctcttcacattttttgtacaaccgacatgcccgtgtagctcacaaatatgacagtggcgtgaattttgcgcattgacggcagttatgattcgcggtattgcttaactgtgattgcacatttagtaatcactgttttcttttccaccagaaaccagtatgagggaaacgaggc

SEQ ID NO: 9 - DNA, 312 bp, synthetic construct
  source 1..312: mol_type = other DNA
gcctgtattcgttgtagtgaaatcattcatatgaaagcgggggaaaaacaattatgtccgcgctgtgcaaatccagaatggacgaaggcaagtcgggcaaaacgggtgacctgacagtaaaaacatcggctttttgctaataatccgagagattcttttgtgtgatgcaagccacatttttgccctcaacggttttactcattgcgatgtgtgtcactgaatgataaaaccgatagccacaggaataatgtattacctgtggtcgcaatcgattgaccgcgggttaatagcaacgcaacgtggtgaggggaa

SEQ ID NO: 10 - DNA, 35 bp, synthetic construct
  source 1..35: mol_type = other DNA
ctgcaggaattcgatgaaggtaaccactttttccg

SEQ ID NO: 11 - DNA, 35 bp, synthetic construct
  source 1..35: mol_type = other DNA
gagttgcagcaagcggaggatcaccacatttttac

SEQ ID NO: 12 - DNA, 35 bp, synthetic construct
  source 1..35: mol_type = other DNA
aatgtggtgatcctccgcttgctgcaactctctca

SEQ ID NO: 13 - DNA, 35 bp, synthetic construct
  source 1..35: mol_type = other DNA
tacgggttcgggcatgatagctctcctgtgtgaaa

SEQ ID NO: 14 - DNA, 35 bp, synthetic construct
  source 1..35: mol_type = other DNA
cacaggagagctatcatgcccgaacccgtagccga

SEQ ID NO: 15 - DNA, 35 bp, synthetic construct
  source 1..35: mol_type = other DNA
gtcgactagcgtgatagcggtttgcctttactggc

SEQ ID NO: 16 - DNA, 20 bp, synthetic construct
  source 1..20: mol_type = other DNA
agttgagcaaaaacgccagt

SEQ ID NO: 17 - DNA, 20 bp, synthetic construct
  source 1..20: mol_type = other DNA
gccataccgtacagccagac

SEQ ID NO: 18 - DNA, 35 bp, synthetic construct
  source 1..35: mol_type = other DNA
ctgcaggaattcgatcaaccaccagagattcacgt

SEQ ID NO: 19 - DNA, 35 bp, synthetic construct
  source 1..35: mol_type = other DNA
gcttcctgactccagtgcttactcatcaaaagtag

SEQ ID NO: 20 - DNA, 35 bp, synthetic construct
  source 1..35: mol_type = other DNA
tgagggaaacgaggcatgagtatgtcaacatccac

SEQ ID NO: 21 - DNA, 35 bp, synthetic construct
  source 1..35: mol_type = other DNA
acggtgagaacgaccgttacatcacgctagtcgac

SEQ ID NO: 22 - DNA, 35 bp, synthetic construct
  source 1..35: mol_type = other DNA
tttgatgagtaagcactggagtcaggaagccgctt

SEQ ID NO: 23 - DNA, 35 bp, synthetic construct
  source 1..35: mol_type = other DNA
tgttgacatactcatgcctcgtttccctcatactg

SEQ ID NO: 24 - DNA, 20 bp, synthetic construct
  source 1..20: mol_type = other DNA
gagagctaccataatccgtg

SEQ ID NO: 25 - DNA, 20 bp, synthetic construct
  source 1..20: mol_type = other DNA
catctcaacgtaacagcagg

SEQ ID NO: 26 - DNA, 35 bp, synthetic construct
  source 1..35: mol_type = other DNA
ctgcaggaattcgataaggattccagtttgcccat

SEQ ID NO: 27 - DNA, 36 bp, synthetic construct
  source 1..36: mol_type = other DNA
gcaatagaagcggcttcctgcttgtgcctctaaaac

SEQ ID NO: 28 - DNA, 30 bp, synthetic construct
  source 1..30: mol_type = other DNA
tgagggaaacgaggcatgacgaactatcgc

SEQ ID NO: 29 - DNA, 35 bp, synthetic construct
  source 1..35: mol_type = other DNA
gtcgactagcgtgatgacaaaaccggcaatagtca

SEQ ID NO: 30 - DNA, 35 bp, synthetic construct
  source 1..35: mol_type = other DNA
ttttagaggcacaagcaggaagccgcttctattgc

SEQ ID NO: 31 - DNA, 35 bp, synthetic construct
  source 1..35: mol_type = other DNA
gcgatagttcgtcatgcctcgtttccctcatactg

SEQ ID NO: 32 - DNA, 35 bp, synthetic construct
  source 1..35: mol_type = other DNA
ctgcaggaattcgatcgttaaaggattccagtttg

SEQ ID NO: 33 - DNA, 35 bp, synthetic construct
  source 1..35: mol_type = other DNA
acaacgaatacaggccttgtgcctctaaaacatag

SEQ ID NO: 34 - DNA, 35 bp, synthetic construct
  source 1..35: mol_type = other DNA
ttttagaggcacaaggcctgtattcgttgtagtga

SEQ ID NO: 35 - DNA, 35 bp, synthetic construct
  source 1..35: mol_type = other DNA
gcgatagttcgtcatttcccctcaccacgttgcgt

SEQ ID NO: 36 - DNA, 35 bp, synthetic construct
  source 1..35: mol_type = other DNA
acgtggtgaggggaaatgacgaactatcgcgttga

SEQ ID NO: 37 - DNA, 35 bp, synthetic construct
  source 1..35: mol_type = other DNA
gtcgactagcgtgatattgacaaaaccggcaatag

SEQ ID NO: 38 - DNA, 35 bp, synthetic construct
  source 1..35: mol_type = other DNA
ctgcaggaattcgataaaggattccagtttgccca

SEQ ID NO: 39 - DNA, 37 bp, synthetic construct
  source 1..37: mol_type = other DNA
gcgacgctcattcaacttgtgcctctaaaacatagcc

SEQ ID NO: 40 - DNA, 36 bp, synthetic construct
  source 1..36: mol_type = other DNA
gttttagaggcacaagttgaatgagcgtcgcatctg

SEQ ID NO: 41 - DNA, 36 bp, synthetic construct
  source 1..36: mol_type = other DNA
gtcgactagcgtgatggttaagtctttttatggcgg

SEQ ID NO: 42 - DNA, 20 bp, synthetic construct
  source 1..20: mol_type = other DNA
tcatacatttctgctatgtt

SEQ ID NO: 43 - DNA, 20 bp, synthetic construct
  source 1..20: mol_type = other DNA
agaggatctgaatcagcatc

SEQ ID NO: 44 - DNA, 20 bp, synthetic construct
  source 1..20: mol_type = other DNA
gtttcttgcgctattctcgg

SEQ ID NO: 45 - protein, 147 aa, unidentified
MSMSTSTEVIAHHWAFAIFLIVAIGLCCLMLVGGWFLGGRARARSKNVPFESGIDSVGSARLRLSAKFYLVAMFFVIFDVEALYLFAWSTSIRESGWVGFVEAAIFIFVLLAGLVYLVRIGALDWTPARSRRERMNPETNSIANRQR

SEQ ID NO: 46 - protein, 220 aa, unidentified
MDYTLTRIDPNGENDRYPLQKQEIVTDPLEQEVNKNVFMGKLNDMVNWGRKNSIWPYNFGLSCCYVEMVTSFTAVHDVARFGAEVLRASPRQADLMVVAGTCFTKMAPVIQRLYDQMLEPKWVISMGACANSGGMYDIYSVVQGVDKFIPVDVYIPGCPPRPEAYMQALMLLQESIGKERRPLSWVVGDQGVYRANMQSERERKRGERIAVTNLRTPDEI

SEQ ID NO: 47 - protein, 600 aa, unidentified
MVNNMTDLTAQEPAWQTRDHLDDPVIGELRNRFGPDAFTVQATRTGVPVVWIKREQLLEVGDFLKKLPKPYVMLFDLHGMDERLRTHREGLPAADFSVFYHLISIDRNRDIMLKVALAENDLHVPTFTKLFPNANWYERETWDLFGITFDGHPNLRRIMMPQTWKGHPLRKDYPARATEFSPFELTKAKQDLEMEALTFKPEEWGMKRGTENEDFMFLNLGPNHPSAHGAFRIVLQLDGEEIVDCVPDIGYHHRGAEKMGERQSWHSYIPYTDRIEYLGGCVNEMPYVLAVEKLAGITVPDRVNVIRVMLSELFRINSHLLYISTFIQDVGAMTPVFFAFTDRQKIYDLVEAITGFRMHPAWFRIGGVAHDLPRGWDRLLREFLDWMPKRLASYEKAALQNTILKGRSQGVAAYGAKEALEWGTTGAGLRATGIDFDVRKARPYSGYENFDFEIPVGGGVSDCYTRVMLKVEELRQSLRILEQCLNNMPEGPFKADHPLTTPPPKERTLQHIETLITHFLQVSWGPVMPANESFQMIEATKGINSYYLTSDGSTMSYRTRVRTPSFAHLQQIPAAIRGSLVSDLIVYLGSIDFVMSDVDR

SEQ ID NO: 48 - protein, 166 aa, unidentified
MHENQQPQTEAFELSAAEREAIEHEMHHYEDPRAASIEALKIVQKQRGWVPDGAIHAIADVLGIPASDVEGVATFYSQIFRQPVGRHVIRYCDSVVCHINGYQGIQAALEKKLNIKPGQTTFDGRFTLLPTCCLGNCDKGPNMMIDEDTHAHLTPEAIPELLERYK

SEQ ID NO: 49 - protein, 445 aa, unidentified
MKNIIRTPETHPLTWRLRDDKQPVWLDEYRSKNGYEGARKALTGLSPDEIVNQVKDAGLKGRGGAGFSTGLKWSLMPKDESMNIRYLLCNADEMEPGTYKDRLLMEQLPHLLVEGMLISAFALKAYRGYIFLRGEYIEAAVNLRRAIAEATEAGLLGKNIMGTGFDFELFVHTGAGRYICGEETALINSLEGRRANPRSKPPFPATSGAWGKPTCVNNVETLCNVPAILANGVEWYQNISKSKDAGTKLMGFSGRVKNPGLWELPFGTTAREILEDYAGGMRDGLKFKAWQPGGAGTDFLTEAHLDLPMEFESIGKAGSRLGTALAMAVDHEINMVSLVRNLEEFFARESCGWCTPCRDGLPWSVKILRALERGEGQPGDIETLEQLCRFLGPGKTFCAHAPGAVEPLQSAIKYFREEFEAGIKQPFSNTHLINGIQPNLLKERW

SEQ ID NO: 50 - protein, 910 aa, unidentified
MLMATIHVDGKEYEVNGADNLLEACLSLGLDIPYFCWHPALGSVGACRQCAVKQYQNAEDTRGRLVMSCMTPASDGTFISIDDEEAKQFRESVVEWLMTNHPHDCPVCEEGGNCHLQDMTVMTGHSFRRYRFTKRTHRNQDLGPFISHEMNRCIACYRCVRYYKDYADGTDLGVYGAHDNVYFGRPEDGTLESEFSGNLVEICPTGVFTDKTHSERYNRKWDMQFAPSICQQCSIGCNISPGERYGELRRIENRYNGTVNHYFLCDRGRFGYGYVNLKDRPRQPVQRRGDDFITLNAEQAMQGAADILRQSKKVIGIGSPRASVESNFALRELVGEENFYTGIAHGEQERLQLALKVLREGGIYTPALREIESYDAVLVLGEDVTQTGARVALAVRQAVKGKAREMAAAQKVADWQIAAILNIGQRAKHPLFVTNVDDTRLDDIAAWTYRAPVEDQARLGFAIAHALDNSAPAVDGIEPELQSKIDVIVQALAGAKKPLIISGTNAGSLEVIQAAANVAKALKGRGADVGITMIARSVNSMGLGIMGGGSLEEALTELETGRADAVVVLENDLHRHASAIRVNAALAKAPLVMVVDHQRTAIMENAHLVLSAASFAESDGTVINNEGRAQRFFQVYDPAYYDSKTVMLESWRWLHSLHSTLLSREVDWTQLDHVIDAVVAKIPELAGIKDAAPDATFRIRGQKLAREPHRYSGRTAMRANISVHEPRQPQDIDTMFTFSMEGNNQPTAHRSQVPFAWAPGWNSPQAWNKFQDEVGGKLRFGDPGVRLFETSENGLDYFTSVPARFQPQDGKWRIAPYYHLFGSDELSQRAPVFQSRMPQPYIKLNPADAAKLGVNAGTRVSFSYDGNTVTLPVEIAEGLTAGQVGLPMGMSGIAPVLAGAHLEDLKEAQQ

SEQ ID NO: 51 - protein, 325 aa, unidentified
MSWISPELIEILLTILKAVVILLVVVTCGAFMSFGERRLLGLFQNRYGPNRVGWGGSLQLVADMIKMFFKEDWIPKFSDRVIFTLAPMIAFTSLLLAFAIVPVSPGWVVADLNIGILFFLMMAGLAVYAVLFAGWSSNNKYSLLGAMRASAQTLSYEVFLGLSLMGVVAQAGSFNMTDIVNSQAHVWNVIPQFFGFITFAIAGVAVCHRHPFDQPEAEQELADGYHIEYSGMKFGLFFVGEYIGIVTISALMVTLFFGGWQGPLLPPFIWFALKTAFFMMMFILIRASLPRPRYDQVMSFGWKICLPLTLINLLVTAAVILWQAQ

SEQ ID NO: 52 - protein, 180 aa, unidentified
MTLKELLVGFGTQVRSIWMIGLHAFAKRETRMYPEEPVYLPPRYRGRIVLTRDPDGEERCVACNLCAVACPVGCISLQKAETKDGRWYPEFFRINFSRCIFCGLCEEACPTTAIQLTPDFEMGEYKRQDLVYEKEDLLISGPGKYPEYNFYRMAGMAIDGKDKGEAENEAKPIDVKSLLP

SEQ ID NO: 53 - protein, 184 aa, unidentified
MEFAFYICGLIAILATLRVITHTNPVHALLYLIISLLAISGVFFSLGAYFAGALEIIVYAGAIMVLFVFVVMMLNLGGSEIEQERQWLKPQVWIGPAILSAIMLVVIVYAILGVNDQGIDGTPISAKAVGITLFGPYVLAVELASMLLLAGLVVAFHVGREERAGEVLSNRKDDSAKRKTEEHA

SEQ ID NO: 54 - protein, 100 aa, unidentified
MIPLQHGLILAAILFVLGLTGLVIRRNLLFMLIGLEIMINASALAFVVAGSYWGQTDGQVMYILAISLAAAEASIGLALLLQLHRRRQNLNIDSVSEMRG

SEQ ID NO: 55 - protein, 613 aa, unidentified
MNMLALTIILPLIGFVLLAFSRGRWSENVSAIVGVGSVGLAALVTAFIGVDFFANGEQTYSQPLWTWMSVGDFNIGFNLVLDGLSLTMLSVVTGVGFLIHMYASWYMRGEEGYSRFFAYTNLFIASMVVLVLADNLLLMYLGWEGVGLCSYLLIGFYYTDPKNGAAAMKAFVVTRVGDVFLAFALFILYNELGTLNFREMVELAPAHFADGNNMLMWATLMLLGGAVGKSAQLPLQTWLADAMAGPTPVSALIHAATMVTAGVYLIARTHGLFLMTPEVLHLVGIVGAVTLLLAGFAALVQTDIKRVLAYSTMSQIGYMFLALGVQAWDAAIFHLMTHAFFKALLFLASGSVILACHHEQNIFKMGGLRKSIPLVYLCFLVGGAALSALPLVTAGFFSKDEILAGAMANGHINLMVAGLVGAFMTSLYTFRMIFIVFHGKEQIHAHAVKGVTHSLPLIVLLILSTFVGALIVPPLQGVLPQTTELAHGSMLTLEITSGVVAVVGILLAAWLWLGKRTLVTSIANSAPGRLLGTWWYNAWGFDWLYDKVFVKPFLGIAWLLKRDPLNSMMNIPAVLSRFAGKGLLLSENGYLRWYVASMSIGAVVVLALLMVLR

SEQ ID NO: 56 - protein, 509 aa, unidentified
MLLPWLILIPFIGGFLCWQTERFGVKVPRWIALITMGLTLALSLQLWLQGGYSLTQSAGIPQWQSEFDMPWIPRFGISIHLAIDGLSLLMVVLTGLLGVLAVLCSWKEIEKYQGFFHLNLMWILGGVIGVFLAIDMFLFFFFWEMMLVPMYFLIALWGHKASDGKTRITAATKFFIYTQASGLVMLIAILALVFVHYNATGVWTFNYEELLNTPMSSGVEYLLMLGFFIAFAVKMPVVPLHGWLPDAHSQAPTAGSVDLAGILLKTAAYGLLRFSLPLFPNASAEFAPIAMWLGVIGIFYGAWMAFAQTDIKRLIAYTSVSHMGFVLIAIYTGSQLAYQGAVIQMIAHGLSAAGLFILCGQLYERIHTRDMRMMGGLWSKMKWLPALSLFFAVATLGMPGTGNFVGEFMILFGSFQVVPVITVISTFGLVFASVYSLAMLHRAYFGKAKSQIASQELPGMSLRELFMILLLVVLLVLLGFYPQPILDTSHSAIGNIQQWFVNSVTTTRP

SEQ ID NO: 57 - protein, 425 aa, unidentified
MDVTPLMRVDGFAMLYTGLVLLASLATCTFAYPWLEGYNDNKDEFYLLVLIAALGGILLANANHLASLFLGIELISLPLFGLVGYAFRQKRSLEASIKYTILSAAASSFLLFGMALVYAQSGDLSFVALGKNLGDGMLNEPLLLAGFGLMIVGLGFKLSLVPFHLWTPDVYQGAPAPVSTFLATASKIAIFGVVMRLFLYAPVGDSEAIRVVLAIIAFASIIFGNLMALSQTNIKRLLGYSSISHLGYLLVALIALQTGEMSMEAVGVYLAGYLFSSLGAFGVVSLMSSPYRGPDADSLFSYRGLFWHRPILAAVMTVMMLSLAGIPMTLGFIGKFYVLAVGVQAHLWWLVGAVVVGSAIGLYYYLRVAVSLYLHAPEQPGRDAPSNWQYSAGGIVVLISALLVLVLGVWPQPLISIVRLAMPLM

SEQ ID NO: 58 - DNA, 4695 bp, synthetic construct
  source 1..4695: mol_type = other DNA
tcgaggccgcgattaaattccaacatggatgctgatttatatgggtataaatgggctcgcgataatgtcgggcaatcaggtgcgacaatctatcgattgtatgggaagcccgatgcgccagagttgtttctgaaacatggcaaaggtagcgttgccaatgatgttacagatgagatggtcagactaaactggctgacggaatttatgcctcttccgaccatcaagcattttatccgtactcctgatgatgcatggttactcaccactgcgatccccgggaaaacagcattccaggtattagaagaatatcctgattcaggtgaaaatattgttgatgcgctggcagtgttcctgcgccggttgcattcgattcctgtttgtaattgtccttttaacagcgatcgcgtatttcgtctcgctcaggcgcaatcacgaatgaataacggtttggttgatgcgagtgattttgatgacgagcgtaatggctggcctgttgaacaagtctggaaagaaatgcataagcttttgccattctcaccggattcagtcgtcactcatggtgatttctcacttgataaccttatttttgacgaggggaaattaataggttgtattgatgttggacgagtcggaatcgcagaccgataccaggatcttgccatcctatggaactgcctcggtgagttttctccttcattacagaaacggctttttcaaaaatatggtattgataatcctgatatgaataaattgcagtttcatttgatgctcgatgagtttttctaatcagaattggttaattggttgtaacactggcagagcattacgctgacttgacgggacggcggctttgttgaataaatcgaacttttgctgagttgaaggatcagatcacgcatcttcccgacaacgcagaccgttccgtggcaaagcaaaagttcaaaatcaccaactggtccacctacaacaaagctctcatcaaccgtggctccctcactttctggctggatgatggggcgattcaggcctggtatgagtcagcaacaccttcttcacgaggcagacctcagcgctcaaagatgcaggggtaaaagctaaccgcatctttaccgacaaggcatccggcagttcaacagatcgggaagggctggatttgctgaggatgaaggtggaggaaggtgatgtcattctggtgaagaagctcgaccgtcttggccgcgacaccgccgacatgatccaactgataaaagagtttgatgctcagggtgtagcggttcggtttattgacgacgggatcagtaccgacggtgatatggggcaaatggtggtcaccgcgcgtaatacgactcactatagggcgaattggagctccaccgcggtggcggccgctctagactttacggtatcgccgctcccgattcgcagcgcatcgccttctatcgccttcttgacgagttcttctgagcgggactctggggttcgctagaggatcgatcctttttaacccatcacatatacctgccgttcactattatttagtgaaatgagatattatgatattttctgaattgtgattaaaaaggcaactttatgcccatgcaacagaaactataaaaaatacagagaatgaaaagaaacagatagattttttagttctttaggcccgtagtctgcaaatccttttatgattttctatcaaacaaaagaggaaaatagaccagttgcaatccaaacgagagtctaatagaatgaggtcgaaaagtaaatcgcgcgggtttgttactgataaagcaggcaagacctaaaatgtgtaaagggcaaagtgtatactttggcgtcaccccttacatattttaggtctttttttattgtgcgtaactaacttgccatcttcaaacaggagggctggaagaagcagaccgctaacacagtacataaaaaaggagacatgaacgatgaacatcaaaaagtttgcaaaacaagcaacagtattaacctttactaccgcactgctggcaggaggcgcaactcaagcgtttgcgaaagaaacgaaccaaaagccatataaggaaacatacggcatttcccatattacacgccatgatatgctgcaaatccctgaacagcaaaaaaatgaaaaatatcaagttcctgaattcgattcgtccacaattaaaaatatctcttctgcaaaaggcctggacgtttgggacagctggccattacaaaacgctgacggcactgtcgcaaactatcacggctaccacatcgtctttgcattagccggagatcctaaaaatgcggatgacacatcgatttacatgttctatcaaaaagtcggcgaaacttctattgacagctggaaaaacgctggccgcgtctttaaagacagcgacaaattcgatgcaaatgattctatcctaaaagaccaaacacaagaatggtcaggttcagccacatttacatctgacggaaaaatccgtttattctacactgatttctccggtaaacattacggcaaacaaacactgacaactgcacaagttaacgtatcagcatcagacagctctttgaacatcaacggtgtagaggattataaatcaatctttgacggtgacggaaaaacgtatcaaaatgtacagcagttcatcgatgaaggcaactacagctcaggcgacaaccatacgctgagagatcctcactacgtagaagataaaggccacaaatacttagtatttgaagcaaacactggaactgaagatggctaccaaggcgaagaatctttatttaacaaagcatactatggcaaaagcacatcattcttccgtcaagaaagtcaaaaacttctgcaaagcgataaaaaacgcacggctgagttagcaaacggcgctctcggtatgattgagctaaacgatgattacacactgaaaaaagtgatgaaaccgctgattgcatctaacacagtaacagatgaaattgaacgcgcgaacgtctttaaaatgaacggcaaatggtacctgttcactgactcccgcggatcaaaaatgacgattgacggcattacgtctaacgatatttacatgcttggttatgtttctaattctttaactggcccatacaagccgctgaacaaaactggccttgtgttaaaaatggatcttgatcctaacgatgtaacctttacttactcacacttcgctgtacctcaagcgaaaggaaacaatgtcgtgattacaagctatatgacaaacagaggattctacgcagacaaacaatcaacgtttgcgccaagcttcctgctgaacatcaaaggcaagaaaacatctgttgtcaaagacagcatccttgaacaaggacaattaacagttaacaaataaaaacgcaaaagaaaatgccgatgggtaccgagcgaaatgaccgaccaagcgacgcccaacctgccatcggatcccccgggctgcaggaattcgatatcacgctagtcgacctagctagcatatggggagatctactagtaaagcatgccaattggtattctatagtgtcacctaaatcgtatgtgtatgatacataaggttatgtattaattgtagccgcgttctaacgacaatatgtacaagcctaattgtgtagcatctggcttactgaagcagaccctatcatctctctcgtaaactgccgtcagagtcggtttggttggacgaaccttctgagtttctggtaacgccgtcccgcacccggaaatggtcagcgaaccaatcagcagggtcatcgctagcccatggctaattcccatgtcagccgttaagtgttcctgtgtcactcaaaattgctttgagaggctctaagggcttctcagtgcgttacatccctggcttgttgtccacaaccgttaaaccttaaaagctttaaaagccttatatattcttttttttcttataaaacttaaaaccttagaggctatttaagttgctgatttatattaattttattgttcaaacatgagagcttagtacgtgaaacatgagagcttagtacgttagccatgagagcttagtacgttagccatgagggtttagttcgttaaacatgagagcttagtacgttaaacatgagagcttagtacgtgaaacatgagagcttagtacgtactatcaacaggttgaactgctgatcttcagatcctctacgccggacgcatcgtggccggatcttgcggccgcaaaaattaaaaatgaagttttaaatcaatctaaagtatatatgagtaaacttggtctgacagttaccaatgcttaatcagtgaggcaccaataactgccttaaaaaaactagcgctgaggtctgcctcgtgaagaaggtgttgctgactcataccaggcctgaatcgccccatcatccagccagaaagtgagggagccacggttgatgagagctttgttgtaggtggaccagttggtgattttgaacttttgctttgccacggaacggtctgcgttgtcgggaagatgcgtgatctgatccttcaactcagcaaaagttcgatttattcaacaaagccacgttgtgtctcaaaatctctgatgttacattgcacaagataaaaatatatcatcatgaacaataaaactgtctgcttacataaacagtaatacaaggggtgttatgagccatattcaacgggaaacgtcttgc

SEQ ID NO: 59 - DNA, 476 bp, synthetic construct
  source 1..476: mol_type = other DNA
cgcttgctgcaactctctcagggccaggcggtgaagggcaatcagctgttgcccgtctcactggtgaaaagaaaaaccaccctggcgcccaatacgcaaaccgcctctccccgcgcgttggccgattcattaatgcagctggcacgacaggtttcccgactggaaagcgggcagtgagcgcaacgcaattaatgtaagttagcgcgaattgatctggtttgacagcttatcatcgactgcacggtgcaccaatgcttctggcgtcaggcagccatcggaagctgtggtatggctgtgcaggtcgtaaatcactgcataattcgtgtcgctcaaggcgcactcccgttctggataatgttttttgcgccgacatcataacggttctggcaaatattctgaaatgagctgttgacaattaatcatccggctcgtataatgtgtggaattgtgagcggataacaatttcacacaggaaa